European Patent Application EP 4 398 255 A2, published July 10, 2024. Title: METHODS, SYSTEMS, AND SOFTWARE FOR IDENTIFYING BIOMOLECULES WITH INTERACTING COMPONENTS. Applicant: CODEXIS, INC. Application EP, filed January 29, 2014. The sequence listing filed with the application follows.

SEQUENCE LISTING (13 sequences)

SEQ ID NO: 1 - protein, 4 aa, synthetic construct
  REGION 1..4: note = Description of Artificial Sequence: Synthetic Peptide
ASGF

SEQ ID NO: 2 - protein, 4 aa, synthetic construct
  REGION 1..4: note = Description of Artificial Sequence: Synthetic Peptide
DFVA

SEQ ID NO: 3 - protein, 4 aa, synthetic construct
  REGION 1..4: note = Description of Artificial Sequence: Synthetic Peptide
KLGA

SEQ ID NO: 4 - protein, 4 aa, synthetic construct
  REGION 1..4: note = Description of Artificial Sequence: Synthetic Peptide
DIVF

SEQ ID NO: 5 - protein, 4 aa, synthetic construct
  REGION 1..4: note = Description of Artificial Sequence: Synthetic Peptide
AIVA

SEQ ID NO: 6 - protein, 4 aa, synthetic construct
  REGION 1..4: note = Description of Artificial Sequence: Synthetic Peptide
DSGF

SEQ ID NO: 7 - protein, 4 aa, synthetic construct
  REGION 1..4: note = Description of Artificial Sequence: Synthetic Peptide
KFGF

SEQ ID NO: 8 - protein, 4 aa, synthetic construct
  REGION 1..4: note = Description of Artificial Sequence: Synthetic Peptide
AFVA

SEQ ID NO: 9 - protein, 4 aa, synthetic construct
  REGION 1..4: note = Description of Artificial Sequence: Synthetic Peptide
KSGF

SEQ ID NO: 10 - protein, 4 aa, synthetic construct
  REGION 1..4: note = Description of Artificial Sequence: Synthetic Peptide
DLVA

SEQ ID NO: 11 - protein, 10 aa, synthetic construct
  REGION 1..10: note = Description of Artificial Sequence: Synthetic Peptide
ILLMGWKCSF

SEQ ID NO: 12 - protein, 10 aa, synthetic construct
  REGION 1..10: note = Description of Artificial Sequence: Synthetic Peptide
VAIPHNRTAY

SEQ ID NO: 13 - protein, 10 aa, synthetic construct
  REGION 1..10: note = Description of Artificial Sequence: Synthetic Peptide
VALPGWKTSF